European Patent Specification EP 3 591 074 B1, published October 23, 2024. Title: Methods for Diagnosing Infectious Disease and Determining HLA Status Using Immune Repertoire Sequencing. Applicant: Adaptive Biotechnologies Corp. Fred Hutchinson Cancer Research Center. The sequence listing filed with the application follows.

SEQUENCE LISTING (163 sequences)

SEQ ID NO: 1 - protein, 13 aa, Homo sapiens
CASSGQGAYEQYF

SEQ ID NO: 2 - protein, 15 aa, Homo sapiens
CASSPDRVGQETQYF

SEQ ID NO: 3 - protein, 15 aa, Homo sapiens
CASSIGPLEHNEQFF

SEQ ID NO: 4 - protein, 13 aa, Homo sapiens
CASSIEGNQPQHF

SEQ ID NO: 5 - protein, 15 aa, Homo sapiens
CASSLVAGGRETQYF

SEQ ID NO: 6 - protein, 13 aa, Homo sapiens
CASSLEAEYEQYF

SEQ ID NO: 7 - protein, 11 aa, Homo sapiens
CATSDGDEQFF

SEQ ID NO: 8 - protein, 16 aa, Homo sapiens
CASSLAPGATNEKLFF

SEQ ID NO: 9 - protein, 13 aa, Homo sapiens
CASSRGRQETQYF

SEQ ID NO: 10 - protein, 15 aa, Homo sapiens
CASSAGQGVTYEQYF

SEQ ID NO: 11 - protein, 12 aa, Homo sapiens
CASSLRREKLFF

SEQ ID NO: 12 - protein, 16 aa, Homo sapiens
CASSLIGVSSYNEQFF

SEQ ID NO: 13 - protein, 15 aa, Homo sapiens
CASSFPTSGQETQYF

SEQ ID NO: 14 - protein, 13 aa, Homo sapiens
CASSPQRNTEAFF

SEQ ID NO: 15 - protein, 13 aa, Homo sapiens
CSVRDNFNQPQHF

SEQ ID NO: 16 - protein, 15 aa, Homo sapiens
CATSRDSQGSYGYTF

SEQ ID NO: 17 - protein, 11 aa, Homo sapiens
CASSPGDEQYF

SEQ ID NO: 18 - protein, 15 aa, Homo sapiens
CASSQTGGRNQPQHF

SEQ ID NO: 19 - protein, 14 aa, Homo sapiens
CASSQNRGQETQYF

SEQ ID NO: 20 - protein, 15 aa, Homo sapiens
CASSLVIGGDTEAFF

SEQ ID NO: 21 - protein, 14 aa, Homo sapiens
CASSFHGFNQPQHF

SEQ ID NO: 22 - protein, 15 aa, Homo sapiens
CASSRLAGGTDTQYF

SEQ ID NO: 23 - protein, 15 aa, Homo sapiens
CASSLPSGLTDTQYF

SEQ ID NO: 24 - protein, 15 aa, Homo sapiens
CATSRDTQGSYGYTF

SEQ ID NO: 25 - protein, 11 aa, Homo sapiens
CATSDGDTQYF

SEQ ID NO: 26 - protein, 15 aa, Homo sapiens
CASSLVASGRETQYF

SEQ ID NO: 27 - protein, 14 aa, Homo sapiens
CASSIWGLDTEAFF

SEQ ID NO: 28 - protein, 11 aa, Homo sapiens
CASSPGDEQFF

SEQ ID NO: 29 - protein, 13 aa, Homo sapiens
CASSPSTGTEAFF

SEQ ID NO: 30 - protein, 14 aa, Homo sapiens
CSVEEDEGIYGYTF

SEQ ID NO: 31 - protein, 13 aa, Homo sapiens
CASSEIPNTEAFF

SEQ ID NO: 32 - protein, 16 aa, Homo sapiens
CASSQVPGQGDNEQFF

SEQ ID NO: 33 - protein, 14 aa, Homo sapiens
CASSPAGLNTEAFF

SEQ ID NO: 34 - protein, 13 aa, Homo sapiens
CASSLGLKGTQYF

SEQ ID NO: 35 - protein, 13 aa, Homo sapiens
CASSGDRLYEQYF

SEQ ID NO: 36 - protein, 13 aa, Homo sapiens
CSVRDNYNQPQHF

SEQ ID NO: 37 - protein, 15 aa, Homo sapiens
CASSYGGLGSYEQYF

SEQ ID NO: 38 - protein, 14 aa, Homo sapiens
CASNRDRGRYEQYF

SEQ ID NO: 39 - protein, 13 aa, Homo sapiens
CASMGGASYEQYF

SEQ ID NO: 40 - protein, 15 aa, Homo sapiens
CASSLGVGPYNEQFF

SEQ ID NO: 41 - protein, 14 aa, Homo sapiens
CASSLGGAGDTQYF

SEQ ID NO: 42 - protein, 14 aa, Homo sapiens
CATSRGTVSYEQYF

SEQ ID NO: 43 - protein, 11 aa, Homo sapiens
CATSDGETQYF

SEQ ID NO: 44 - protein, 15 aa, Homo sapiens
CASSEARGGVEKLFF

SEQ ID NO: 45 - protein, 14 aa, Homo sapiens
CASSLNRGQETQYF

SEQ ID NO: 46 - protein, 13 aa, Homo sapiens
CSVRDNHNQPQHF

SEQ ID NO: 47 - protein, 15 aa, Homo sapiens
CASSESGHRNQPQHF

SEQ ID NO: 48 - protein, 15 aa, Homo sapiens
CSASPGQGASYGYTF

SEQ ID NO: 49 - protein, 12 aa, Homo sapiens
CASSEARTRAFF

SEQ ID NO: 50 - protein, 12 aa, Homo sapiens
CASRPTGYEQYF

SEQ ID NO: 51 - protein, 14 aa, Homo sapiens
CASSVTGGTDTQYF

SEQ ID NO: 52 - protein, 15 aa, Homo sapiens
CASSRLAASTDTQYF

SEQ ID NO: 53 - protein, 15 aa, Homo sapiens
CATSDSVTNTGELFF

SEQ ID NO: 54 - protein, 15 aa, Homo sapiens
CASSRNRESNQPQHF

SEQ ID NO: 55 - protein, 13 aa, Homo sapiens
CASSAQGAYEQYF

SEQ ID NO: 56 - protein, 15 aa, Homo sapiens
CASSIQGYSNQPQHF

SEQ ID NO: 57 - protein, 15 aa, Homo sapiens
CASSYNPYSNQPQHF

SEQ ID NO: 58 - protein, 17 aa, Homo sapiens
CASSLGHRDPNTGELFF

SEQ ID NO: 59 - protein, 13 aa, Homo sapiens
CASSTTGGDGYTF

SEQ ID NO: 60 - protein, 15 aa, Homo sapiens
CASSVLAGPTDTQYF

SEQ ID NO: 61 - protein, 12 aa, Homo sapiens
CASSYRQETQYF

SEQ ID NO: 62 - protein, 13 aa, Homo sapiens
CASSSGQVYGYTF

SEQ ID NO: 63 - protein, 12 aa, Homo sapiens
CASGRDTYEQYF

SEQ ID NO: 64 - protein, 16 aa, Homo sapiens
CATSDSRTGGQETQYF

SEQ ID NO: 65 - protein, 16 aa, Homo sapiens
CASSSPGRSGANVLTF

SEQ ID NO: 66 - protein, 12 aa, Homo sapiens
CASSYGGEGYTF

SEQ ID NO: 67 - protein, 14 aa, Homo sapiens
CASSLAGVDYEQYF

SEQ ID NO: 68 - protein, 13 aa, Homo sapiens
CASSLQGADTQYF

SEQ ID NO: 69 - protein, 13 aa, Homo sapiens
CASSLEAENEQFF

SEQ ID NO: 70 - protein, 16 aa, Homo sapiens
CASSEAPSTSTDTQYF

SEQ ID NO: 71 - protein, 13 aa, Homo sapiens
CASSLEGQQPQHF

SEQ ID NO: 72 - protein, 16 aa, Homo sapiens
CASSLGHRDSSYEQYF

SEQ ID NO: 73 - protein, 13 aa, Homo sapiens
CASSPSRNTEAFF

SEQ ID NO: 74 - protein, 13 aa, Homo sapiens
CSALGHSNQPQHF

SEQ ID NO: 75 - protein, 14 aa, Homo sapiens
CASSHRDRNYEQYF

SEQ ID NO: 76 - protein, 15 aa, Homo sapiens
CASSPPGQGSDTQYF

SEQ ID NO: 77 - protein, 15 aa, Homo sapiens
CASSLQGYSNQPQHF

SEQ ID NO: 78 - protein, 16 aa, Homo sapiens
CASSYVRTGGNYGYTF

SEQ ID NO: 79 - protein, 13 aa, Homo sapiens
CASSRDRNYGYTF

SEQ ID NO: 80 - protein, 15 aa, Homo sapiens
CASSTGTSGSYEQYF

SEQ ID NO: 81 - protein, 14 aa, Homo sapiens
CASRSDSGANVLTF

SEQ ID NO: 82 - protein, 13 aa, Homo sapiens
CATSRVAGETQYF

SEQ ID NO: 83 - protein, 13 aa, Homo sapiens
CASSEEGIQPQHF

SEQ ID NO: 84 - protein, 14 aa, Homo sapiens
CASSLGGPGDTQYF

SEQ ID NO: 85 - protein, 15 aa, Homo sapiens
CASSLVAAGRETQYF

SEQ ID NO: 86 - protein, 14 aa, Homo sapiens
CASRGQGWDEKLFF

SEQ ID NO: 87 - protein, 14 aa, Homo sapiens
CASSLEGQGFGYTF

SEQ ID NO: 88 - protein, 14 aa, Homo sapiens
CASRDWDYTDTQYF

SEQ ID NO: 89 - protein, 17 aa, Homo sapiens
CASSRSGLAGNTGELFF

SEQ ID NO: 90 - protein, 16 aa, Homo sapiens
CASSPGQEAGANVLTF

SEQ ID NO: 91 - protein, 14 aa, Homo sapiens
CASSLGDRPDTQYF

SEQ ID NO: 92 - protein, 13 aa, Homo sapiens
CASSFPGGETQYF

SEQ ID NO: 93 - protein, 12 aa, Homo sapiens
CASSLETYGYTF

SEQ ID NO: 94 - protein, 14 aa, Homo sapiens
CASSSGQVQETQYF

SEQ ID NO: 95 - protein, 12 aa, Homo sapiens
CASSFDNYGYTF

SEQ ID NO: 96 - protein, 13 aa, Homo sapiens
CASSEGARQPQHF

SEQ ID NO: 97 - protein, 15 aa, Homo sapiens
CASSLTGGRNQPQHF

SEQ ID NO: 98 - protein, 13 aa, Homo sapiens
CASSLLWDQPQHF

SEQ ID NO: 99 - protein, 16 aa, Homo sapiens
CASSLFGTGGNTEAFF

SEQ ID NO: 100 - protein, 12 aa, Homo sapiens
CASSISAGEAFF

SEQ ID NO: 101 - protein, 15 aa, Homo sapiens
CASSPPSGLTDTQYF

SEQ ID NO: 102 - protein, 12 aa, Homo sapiens
CASSPLSDTQYF

SEQ ID NO: 103 - protein, 13 aa, Homo sapiens
CASSSRGTGELFF

SEQ ID NO: 104 - protein, 12 aa, Homo sapiens
CASSYAGDGYTF

SEQ ID NO: 105 - protein, 14 aa, Homo sapiens
CASSDRGNTGELFF

SEQ ID NO: 106 - protein, 11 aa, Homo sapiens
CASSPGGTQYF

SEQ ID NO: 107 - protein, 15 aa, Homo sapiens
CASSLGDRAYNEQFF

SEQ ID NO: 108 - protein, 15 aa, Homo sapiens
CASSLRGSSYNEQFF

SEQ ID NO: 109 - protein, 14 aa, Homo sapiens
CASSLTASSYEQYF

SEQ ID NO: 110 - protein, 10 aa, Homo sapiens
CSASDHEQYF

SEQ ID NO: 111 - protein, 14 aa, Homo sapiens
CASSQGRHTDTQYF

SEQ ID NO: 112 - protein, 15 aa, Homo sapiens
CASSRPGQGNTEAFF

SEQ ID NO: 113 - protein, 12 aa, Homo sapiens
CASSLVGDGYTF

SEQ ID NO: 114 - protein, 14 aa, Homo sapiens
CASSLGAGNQPQHF

SEQ ID NO: 115 - protein, 13 aa, Homo sapiens
CASSLTDTGELFF

SEQ ID NO: 116 - protein, 16 aa, Homo sapiens
CASSLTGGNSGNTIYF

SEQ ID NO: 117 - protein, 13 aa, Homo sapiens
CAWRGTGNSPLHF

SEQ ID NO: 118 - protein, 12 aa, Homo sapiens
CASASANYGYTF

SEQ ID NO: 119 - protein, 14 aa, Homo sapiens
CASSLQAGANEQFF

SEQ ID NO: 120 - protein, 14 aa, Homo sapiens
CASSEEAGGSGYTF

SEQ ID NO: 121 - protein, 12 aa, Homo sapiens
CASRTGESGYTF

SEQ ID NO: 122 - protein, 11 aa, Homo sapiens
CASSGLNEQFF

SEQ ID NO: 123 - protein, 14 aa, Homo sapiens
CASSWDRDNSPLHF

SEQ ID NO: 124 - protein, 14 aa, Homo sapiens
CASSIRTNYYGYTF

SEQ ID NO: 125 - protein, 10 aa, Homo sapiens
CSARSPEAFF

SEQ ID NO: 126 - protein, 15 aa, Homo sapiens
CASSRGTGATDTQYF

SEQ ID NO: 127 - protein, 14 aa, Homo sapiens
CASSPRVSNQPQHF

SEQ ID NO: 128 - protein, 15 aa, Homo sapiens
CAISESQDRGHEQYF

SEQ ID NO: 129 - protein, 14 aa, Homo sapiens
CASSLGRGYEKLFF

SEQ ID NO: 130 - protein, 13 aa, Homo sapiens
CSVEVRGTDTQYF

SEQ ID NO: 131 - protein, 13 aa, Homo sapiens
CASRGQGAGELFF

SEQ ID NO: 132 - protein, 14 aa, Homo sapiens
CATSREGSGYEQYF

SEQ ID NO: 133 - protein, 12 aa, Homo sapiens
CASSLGWTEAFF

SEQ ID NO: 134 - protein, 15 aa, Homo sapiens
CASSLGSSSYNEQFF

SEQ ID NO: 135 - protein, 13 aa, Homo sapiens
CASSSAGADTQYF

SEQ ID NO: 136 - protein, 13 aa, Homo sapiens
CASSERKNYGYTF

SEQ ID NO: 137 - protein, 15 aa, Homo sapiens
CASRDRDRVNTEAFF

SEQ ID NO: 138 - protein, 11 aa, Homo sapiens
CASSRVGEQFF

SEQ ID NO: 139 - protein, 13 aa, Homo sapiens
CASSPRWQETQYF

SEQ ID NO: 140 - protein, 11 aa, Homo sapiens
CASTPGDTIYF

SEQ ID NO: 141 - protein, 14 aa, Homo sapiens
CASSENGGNQPQHF

SEQ ID NO: 142 - protein, 12 aa, Homo sapiens
CASSYPGETQYF

SEQ ID NO: 143 - DNA, 39 bp, Homo sapiens
tgtgccagcagtgggggggcaaacaccgggcagctctac

SEQ ID NO: 144 - DNA, 12 bp, Homo sapiens
agtgggggggca

SEQ ID NO: 145 - DNA, 39 bp, Homo sapiens
tgtgccagcagtgggggggcgaacaccgggcagctctac

SEQ ID NO: 146 - DNA, 12 bp, Homo sapiens
agtgggggggcg

SEQ ID NO: 147 - DNA, 39 bp, Homo sapiens
tgtgccagcagcgggggggcaaacaccgggcagctctac

SEQ ID NO: 148 - DNA, 12 bp, Homo sapiens
agcgggggggca

SEQ ID NO: 149 - protein, 13 aa, Homo sapiens
CASSGGANTGQLY

SEQ ID NO: 150 - protein, 14 aa, Homo sapiens
CASSLEAGAQPQHF

SEQ ID NO: 151 - protein, 13 aa, Homo sapiens
CASSIRSGVEQYF

SEQ ID NO: 152 - protein, 14 aa, Homo sapiens
CSARDRGIGNTIYF

SEQ ID NO: 153 - protein, 13 aa, Homo sapiens
CASSQSPGGTQYF

SEQ ID NO: 154 - protein, 12 aa, Homo sapiens
CASSPETGEAFF

SEQ ID NO: 155 - protein, 13 aa, Homo sapiens
CASSLRSTGELFF

SEQ ID NO: 156 - protein, 14 aa, Homo sapiens
CASSENSPHQPQHF

SEQ ID NO: 157 - protein, 12 aa, Homo sapiens
CASSQEAGPQHF

SEQ ID NO: 158 - protein, 14 aa, Homo sapiens
CASSIRDRGQPQHF

SEQ ID NO: 159 - protein, 13 aa, Homo sapiens
CASSYQGGNEQFF

SEQ ID NO: 160 - protein, 12 aa, Homo sapiens
CASSGGANVLTF

SEQ ID NO: 161 - protein, 12 aa, Homo sapiens
CSVEDLGYGYTF

SEQ ID NO: 162 - protein, 15 aa, Homo sapiens
CASRRGGSSYNEQFF

SEQ ID NO: 163 - protein, 11 aa, Homo sapiens
CASRSGTEAFF